European Patent Application EP 4 151 743 A1, published March 22, 2023. Title: HIGH REBAUDIOSIDE M CONTENT RATIO STEVIA PLANT AND SCREENING METHOD THEREFOR. Applicant: SUNTORY HOLDINGS LIMITED. The sequence listing filed with the application follows.

SEQUENCE LISTING (110 sequences)

SEQ ID NO: 1 - DNA, 326 bp, Stevia rebaudiana
ggcagccattgatgatgttgttgaatgtgattaatttgaatgttataaagaatttggaaaagaaaaaggaggggacaaagttgatgaaattaggggagttatgattatgatggccatggtgattgtgatgagtggcactatgtaatctaatatttgaagatatgagaccacttgaccatgttataatcttatacaaaataattaatccctcacggtaatttttttctaatccttaaactgaaatttgaaagtaatttgagatagtgtttcccctaatttatgcttttagtatgcatttattctatcatattttctatgagaattgg

SEQ ID NO: 2 - DNA, 70 bp, Stevia rebaudiana
tgattttgaaaggatctgactgtatgtttataagacatagttatgagtttgaaccccaatggctaaccct

SEQ ID NO: 3 - DNA, 383 bp, Stevia rebaudiana
aaggttctttatttttaaacttatgttaatttattgtatcttgtagttaatcaagagatgctctcttggagaaattttatggtcataaaacctatatcaaagagatgctctcttggtatattccatacttaaaatatctattttggaaaaaaagtgtagcatcttcctgcttttagtaggtgtcaatcattattaaatttcacaaaaccgtgcaagaatcccagtttccctatagtttgtatacgttcctgatctagtattttacttatgtttcaaatcaatccaatcatgcttgtgtccgaaaattaaaaaacaagggtattggatgccctgtaccactattattaacttttcagaaaaacgtgtagcatgtgtacataagg

SEQ ID NO: 4 - DNA, 297 bp, Stevia rebaudiana
taatcatccaaaccctaatctcgccaaacaaccgaatactgatccaaaccctgaaatgagcacaactcttgaacctgatcacgagaatgaagagcacaaacatgttatgacacatgtaaacgatggtttttgctacatgaaaaccctagaagacgaaacccgtttaactgtaaatcttgaaaacacattctttgatgaaaaacccctttcgtatccggatcttatggacttttctgcatcgaaaacggacgaatacgacttctatgatgaacttgaagagctgccaatgtcttcctc

SEQ ID NO: 5 - DNA, 390 bp, Stevia rebaudiana
cgatggtttttgctacatgaaaaccctagaagacgaaacccgtttaactgtaaatcttgaaaacacattctttgatgaaaaacccctttcgtatccggatcttatggacttttctgcatcgaaaacggacgaatacgacttctatgatgaacttgaagagctgccaatgtcttcctcatcattcaaaagcttcatgagaagtaatttctttgaggaaagagttcttgttcaaccttattgattaagaatttaagggaagcagattatatatgtaattaaattttggtatttatactttgaacttaattaataattataataataatcccaactagaggcacttagtggagattacttatatataatactaattcaaggattattgctggt

SEQ ID NO: 6 - DNA, 158 bp, Stevia rebaudiana
cgcaaacacgtatactaatcacgtaacatattttttatttctaaattaaaattttataacaatatcatacttgaattaaagataacataatatttatttttagagtgtaacttctaaaaaatatcaacctacgaaaaagttgtacataccatgctaaa

SEQ ID NO: 7 - DNA, 288 bp, Stevia rebaudiana
atacaaaaacacaacccatatggtcaaatcaacccattcatgagtaatcaggtcaaattcgctatctgagctgatgcattcaactatttggtctctttttaacatttattttttttattattttgaatgtagaaactttggaactactcaactggtaagttcttgaagatgtataccggtcatgtaaacaaaacatattgtataactccgactttttctgtaacaaatggaaaatatattgttagtggttcagaagatcattgtgtctacatatgggatttacaaggg

SEQ ID NO: 8 - DNA, 25 bp, Artificial Sequence
  Synthetic DNA
ggcagccattgatgatgttgttgaa

SEQ ID NO: 9 - DNA, 36 bp, Artificial Sequence
  Synthetic DNA
ccaattctcatagaaaatatgatagaataaatgcat

SEQ ID NO: 10 - DNA, 32 bp, Artificial Sequence
  Synthetic DNA
tgattttgaaaggatctgactgtatgtttata

SEQ ID NO: 11 - DNA, 20 bp, Artificial Sequence
  Synthetic DNA
agggttagccattggggttc

SEQ ID NO: 12 - DNA, 43 bp, Artificial Sequence
  Synthetic DNA
aaggttctttatttttaaacttatgttaatttattgtatcttg

SEQ ID NO: 13 - DNA, 21 bp, Artificial Sequence
  Synthetic DNA
ccttatgtacacatgctacac

SEQ ID NO: 14 - DNA, 39 bp, Artificial Sequence
  Synthetic DNA
taatcatccaaaccctaatctcgccaaacaaccgaatac

SEQ ID NO: 15 - DNA, 20 bp, Artificial Sequence
  Synthetic DNA
gaggaagacattggcaactc

SEQ ID NO: 16 - DNA, 47 bp, Artificial Sequence
  Synthetic DNA
cgatggtttttgctacatgaaaaccctagaagacgaaacccgtttaa

SEQ ID NO: 17 - DNA, 23 bp, Artificial Sequence
  Synthetic DNA
accagcaataatccttgaattag

SEQ ID NO: 18 - DNA, 20 bp, Artificial Sequence
  Synthetic DNA
cgcaaacacgtatactaatc

SEQ ID NO: 19 - DNA, 20 bp, Artificial Sequence
  Synthetic DNA
tttagcatggtatgtacaac

SEQ ID NO: 20 - DNA, 49 bp, Artificial Sequence
  Synthetic DNA
atacaaaaacacaacccatatggtcaaatcaacccattcatgagtaatc

SEQ ID NO: 21 - DNA, 22 bp, Artificial Sequence
  Synthetic DNA
cccttgtaaatcccatatgtag

SEQ ID NO: 22 - DNA, 21 bp, Stevia rebaudiana
atgcttttagtatgcatttat

SEQ ID NO: 23 - DNA, 41 bp, Stevia rebaudiana
cccctaatttatgcttttagtatgcatttattctatcatat

SEQ ID NO: 24 - DNA, 61 bp, Stevia rebaudiana
gatagtgtttcccctaatttatgcttttagtatgcatttattctatcatattttctatgag

SEQ ID NO: 25 - DNA, 21 bp, Stevia rebaudiana
tatgtttataagacatagtta

SEQ ID NO: 26 - DNA, 41 bp, Stevia rebaudiana
gatctgactgtatgtttataagacatagttatgagtttgaa

SEQ ID NO: 27 - DNA, 61 bp, Stevia rebaudiana
attttgaaaggatctgactgtatgtttataagacatagttatgagtttgaaccccaatggc

SEQ ID NO: 28 - DNA, 21 bp, Stevia rebaudiana
ttgtatcttgtagttaatcaa

SEQ ID NO: 29 - DNA, 41 bp, Stevia rebaudiana
tgttaatttattgtatcttgtagttaatcaagagatgctct

SEQ ID NO: 30 - DNA, 61 bp, Stevia rebaudiana
tttaaacttatgttaatttattgtatcttgtagttaatcaagagatgctctcttggagaaa

SEQ ID NO: 31 - DNA, 21 bp, Stevia rebaudiana
aaccgaatactgatccaaacc

SEQ ID NO: 32 - DNA, 41 bp, Stevia rebaudiana
ctcgccaaacaaccgaatactgatccaaaccctgaaatgag

SEQ ID NO: 33 - DNA, 61 bp, Stevia rebaudiana
aaaccctaatctcgccaaacaaccgaatactgatccaaaccctgaaatgagcacaactctt

SEQ ID NO: 34 - DNA, 21 bp, Stevia rebaudiana
acccgtttaactgtaaatctt

SEQ ID NO: 35 - DNA, 41 bp, Stevia rebaudiana
agaagacgaaacccgtttaactgtaaatcttgaaaacacat

SEQ ID NO: 36 - DNA, 61 bp, Stevia rebaudiana
tgaaaaccctagaagacgaaacccgtttaactgtaaatcttgaaaacacattctttgatga

SEQ ID NO: 37 - DNA, 20 bp, Stevia rebaudiana
attaaaatttgaattaaaga

SEQ ID NO: 38 - DNA, 40 bp, Stevia rebaudiana
ttatttctaaattaaaatttgaattaaagataacataata

SEQ ID NO: 39 - DNA, 60 bp, Stevia rebaudiana
aacatattttttatttctaaattaaaatttgaattaaagataacataatatttattttta

SEQ ID NO: 40 - DNA, 21 bp, Stevia rebaudiana
atgagtaatcaggtcaaattc

SEQ ID NO: 41 - DNA, 41 bp, Stevia rebaudiana
caacccattcatgagtaatcaggtcaaattcgctatctgag

SEQ ID NO: 42 - DNA, 61 bp, Stevia rebaudiana
atggtcaaatcaacccattcatgagtaatcaggtcaaattcgctatctgagctgatgcatt

SEQ ID NO: 43 - DNA, 25 bp, Artificial Sequence
  Synthetic DNA
ggcagccattgatgatgttgttgaa

SEQ ID NO: 44 - DNA, 36 bp, Artificial Sequence
  Synthetic DNA
ccaattctcatagaaaatatgatagaataaatgcgt

SEQ ID NO: 45 - DNA, 326 bp, Artificial Sequence
  Synthetic DNA
ggcagccattgatgatgttgttgaatgtgattaatttgaatgttataaagaatttggaaaagaaaaaggaggggacaaagttgatgaaattaggggagttatgattatgatggccatggtgattgtgatgagtggcactatgtaatctaatatttgaagatatgagaccacttgaccatgttataatcttatacaaaataattaatccctcacggtaatttttttctaatccttaaactgaaatttgaaagtaatttgagatagtgtttcccctaatttatgcttttagtacgcatttattctatcatattttctatgagaattgg

SEQ ID NO: 46 - DNA, 290 bp, Artificial Sequence
  Synthetic DNA
ggcagccattgatgatgttgttgaatgtgattaatttgaatgttataaagaatttggaaaagaaaaaggaggggacaaagttgatgaaattaggggagttatgattatgatggccatggtgattgtgatgagtggcactatgtaatctaatatttgaagatatgagaccacttgaccatgttataatcttatacaaaataattaatccctcacggtaatttttttctaatccttaaactgaaatttgaaagtaatttgagatagtgtttcccctaatttatgcttttagt

SEQ ID NO: 47 - DNA, 36 bp, Artificial Sequence
  Synthetic DNA
acgcatttattctatcatattttctatgagaattgg

SEQ ID NO: 48 - DNA, 326 bp, Artificial Sequence
  Synthetic DNA
ggcagccattgatgatgttgttgaatgtgattaatttgaatgttataaagaatttggaaaagaaaaaggaggggacaaagttgatgaaattaggggagttatgattatgatggccatggtgattgtgatgagtggcactatgtaatctaatatttgaagatatgagaccacttgaccatgttataatcttatacaaaataattaatccctcacggtaatttttttctaatccttaaactgaaatttgaaagtaatttgagatagtgtttcccctaatttatgcttttagcacgcatttattctatcatattttctatgagaattgg

SEQ ID NO: 49 - DNA, 32 bp, Artificial Sequence
  Synthetic DNA
tgattttgaaaggatctgactgtatgttttta

SEQ ID NO: 50 - DNA, 20 bp, Artificial Sequence
  Synthetic DNA
tgttgaccatcaagccacat

SEQ ID NO: 51 - DNA, 196 bp, Artificial Sequence
  Synthetic DNA
tgattttgaaaggatctgactgtatgtttttaagacatagttatgagtttgaaccccaatggctaacccttttagagaagctccatcacctaccggtggttcctgtcggattattgccaccagaaaaacccaccaacatcgaagacgggaatgatgagacgtgggacacagtcaagatgtggcttgatggtcaaca

SEQ ID NO: 52 - DNA, 30 bp, Artificial Sequence
  Synthetic DNA
tgattttgaaaggatctgactgtatgtttt

SEQ ID NO: 53 - DNA, 166 bp, Artificial Sequence
  Synthetic DNA
taagacatagttatgagtttgaaccccaatggctaacccttttagagaagctccatcacctaccggtggttcctgtcggattattgccaccagaaaaacccaccaacatcgaagacgggaatgatgagacgtgggacacagtcaagatgtggcttgatggtcaaca

SEQ ID NO: 54 - DNA, 196 bp, Artificial Sequence
  Synthetic DNA
tgattttgaaaggatctgactgtatgtttttatgacatagttatgagtttgaaccccaatggctaacccttttagagaagctccatcacctaccggtggttcctgtcggattattgccaccagaaaaacccaccaacatcgaagacgggaatgatgagacgtgggacacagtcaagatgtggcttgatggtcaaca

SEQ ID NO: 55 - DNA, 43 bp, Artificial Sequence
  Synthetic DNA
aaggttctttatttttaaacttatgttaatttattgtatctag

SEQ ID NO: 56 - DNA, 21 bp, Artificial Sequence
  Synthetic DNA
ccttatgtacacatgctacac

SEQ ID NO: 57 - DNA, 383 bp, Artificial Sequence
  Synthetic DNA
aaggttctttatttttaaacttatgttaatttattgtatctagtagttaatcaagagatgctctcttggagaaattttatggtcataaaacctatatcaaagagatgctctcttggtatattccatacttaaaatatctattttggaaaaaaagtgtagcatcttcctgcttttagtaggtgtcaatcattattaaatttcacaaaaccgtgcaagaatcccagtttccctatagtttgtatacgttcctgatctagtattttacttatgtttcaaatcaatccaatcatgcttgtgtccgaaaattaaaaaacaagggtattggatgccctgtaccactattattaacttttcagaaaaacgtgtagcatgtgtacataagg

SEQ ID NO: 58 - DNA, 383 bp, Artificial Sequence
  Synthetic DNA
aaggttctttatttttaaacttatgttaatttattgtatctagaagttaatcaagagatgctctcttggagaaattttatggtcataaaacctatatcaaagagatgctctcttggtatattccatacttaaaatatctattttggaaaaaaagtgtagcatcttcctgcttttagtaggtgtcaatcattattaaatttcacaaaaccgtgcaagaatcccagtttccctatagtttgtatacgttcctgatctagtattttacttatgtttcaaatcagtccaatcatgcttgtgtccgaaaattaaaaaacaagggtattggatgccctgtaccactattattaacttttcagaaaaacgtgtagcatgtgtacataagg

SEQ ID NO: 59 - DNA, 344 bp, Artificial Sequence
  Synthetic DNA
ctagaagttaatcaagagatgctctcttggagaaattttatggtcataaaacctatatcaaagagatgctctcttggtatattccatacttaaaatatctattttggaaaaaaagtgtagcatcttcctgcttttagtaggtgtcaatcattattaaatttcacaaaaccgtgcaagaatcccagtttccctatagtttgtatacgttcctgatctagtattttacttatgtttcaaatcagtccaatcatgcttgtgtccgaaaattaaaaaacaagggtattggatgccctgtaccactattattaacttttcagaaaaacgtgtagcatgtgtacataagg

SEQ ID NO: 60 - DNA, 39 bp, Artificial Sequence
  Synthetic DNA
taatcatccaaaccctaatctcgccaaacaaccgggtac

SEQ ID NO: 61 - DNA, 20 bp, Artificial Sequence
  Synthetic DNA
gaggaagacattggcaactc

SEQ ID NO: 62 - DNA, 297 bp, Artificial Sequence
  Synthetic DNA
taatcatccaaaccctaatctcgccaaacaaccgggtactgatccaaaccctgaaatgagcacaactcttgaacctgatcacgagaatgaagagcacaaacatgttatgacacatgtaaacgatggtttttgctacatgaaaaccctagaagacgaaacccgtttaactgtaaatcttgaaaacacattctttgatgaaaaacccctttcgtatccggatcttatggacttttctgcatcgaaaacggacgaatacgacttctatgatgaacttgaagagctgccaatgtcttcctc

SEQ ID NO: 63 - DNA, 297 bp, Artificial Sequence
  Synthetic DNA
taatcatccaaaccctaatctcgccaaacaaccgggtaccgatccaaaccctgaaatgagcacaactcttgaacctgatcacgagaatgaagagcacaaacatgttatgacacatgtaaacgatggtttttgctacatgaaaaccctagaagacgaaacccgtttaagtgtaaatcttgaaaacacattctttgatgaagaacccctttcgtatccggatcttatggacttttctgcatcgaaaaaggacgaatacgacttctatgatgaacttgaagagttgccaatgtcttcctc

SEQ ID NO: 64 - DNA, 258 bp, Artificial Sequence
  Synthetic DNA
cgatccaaaccctgaaatgagcacaactcttgaacctgatcacgagaatgaagagcacaaacatgttatgacacatgtaaacgatggtttttgctacatgaaaaccctagaagacgaaacccgtttaagtgtaaatcttgaaaacacattctttgatgaagaacccctttcgtatccggatcttatggacttttctgcatcgaaaaaggacgaatacgacttctatgatgaacttgaagagttgccaatgtcttcctc

SEQ ID NO: 65 - DNA, 47 bp, Artificial Sequence
  Synthetic DNA
cgatggtttttgctacatgaaaaccctagaagacgaaacccgcttaa

SEQ ID NO: 66 - DNA, 23 bp, Artificial Sequence
  Synthetic DNA
accagcaataatccttgaattag

SEQ ID NO: 67 - DNA, 390 bp, Artificial Sequence
  Synthetic DNA
cgatggtttttgctacatgaaaaccctagaagacgaaacccgcttaactgtaaatcttgaaaacacattctttgatgaaaaacccctttcgtatccggatcttatggacttttctgcatcgaaaacggacgaatacgacttctatgatgaacttgaagagctgccaatgtcttcctcatcattcaaaagcttcatgagaagtaatttctttgaggaaagagttcttgttcaaccttattgattaagaatttaagggaagcagattatatatgtaattaaattttggtatttatactttgaacttaattaataattataataataatcccaactagaggcacttagtggagattacttatatataatactaattcaaggattattgctggt

SEQ ID NO: 68 - DNA, 390 bp, Artificial Sequence
  Synthetic DNA
cgatggtttttgctacatgaaaaccctagaagacgaaacccgcttaagtgtaaatcttgaaaacacattctttgatgaagaacccctttcgtatccggatcttatggacttttctgcatcgaaaaaggacgaatacgacttctatgatgaacttgaagagttgccaatgtcttcctcatcattcaaaagcttcatgagaagtaatttctttgaggaaagagttcttgttcaaccttattgattaagaatttaagggaagcagattatatatgtaattaaattttggtatttatactttgaacttaattaataattataataataatcccaactagaggcacttagtggagattacttatatataatactaattcaaggattattgctggt

SEQ ID NO: 69 - DNA, 347 bp, Artificial Sequence
  Synthetic DNA
ttaagtgtaaatcttgaaaacacattctttgatgaagaacccctttcgtatccggatcttatggacttttctgcatcgaaaaaggacgaatacgacttctatgatgaacttgaagagttgccaatgtcttcctcatcattcaaaagcttcatgagaagtaatttctttgaggaaagagttcttgttcaaccttattgattaagaatttaagggaagcagattatatatgtaattaaattttggtatttatactttgaacttaattaataattataataataatcccaactagaggcacttagtggagattacttatatataatactaattcaaggattattgctggt

SEQ ID NO: 70 - DNA, 20 bp, Artificial Sequence
  Synthetic DNA
cgcaaacacgtatactaatc

SEQ ID NO: 71 - DNA, 20 bp, Artificial Sequence
  Synthetic DNA
tttagcatggtatgtacaac

SEQ ID NO: 72 - DNA, 140 bp, Artificial Sequence
  Synthetic DNA
cgcaaacacgtatactaatcacgtaacatattttttatttctaaattaaaatttgaattaaagataacataatatttatttttagagtgtaacttctaaaaaatatcaacctacgaaaaagttgtacataccatgctaaa

SEQ ID NO: 73 - DNA, 158 bp, Artificial Sequence; identical to SEQ ID NO: 6
  Synthetic DNA

SEQ ID NO: 74 - DNA, 49 bp, Artificial Sequence
  Synthetic DNA
atacaaaaacacaacccatatggtcaaatcaacccattcatgagcgatc

SEQ ID NO: 75 - DNA, 22 bp, Artificial Sequence
  Synthetic DNA
cccttgtaaatcccatatgtag

SEQ ID NO: 76 - DNA, 288 bp, Artificial Sequence
  Synthetic DNA
atacaaaaacacaacccatatggtcaaatcaacccattcatgagcgatcaggtcaaattcgctatctgagctgatgcattcaactatttggtctctttttaacatttattttttttattattttgaatgtagaaactttggaactactcaactggtaagttcttgaagatgtataccggtcatgtaaacaaaacatattgtataactccgactttttctgtaacaaatggaaaatatattgttagtggttcagaagatcattgtgtctacatatgggatttacaaggg

SEQ ID NO: 77 - DNA, 288 bp, Artificial Sequence
  Synthetic DNA
atacaaaaacacaacccatatggtcaaatcaacccattcatgagcgatcgggtcaaattcgctatctgagctgatgcattcaactatttggtctctttttaacatttattttttttattattttgaatgtagaaactttggaactactcaactggtaagttcttgaagatgtataccggtcatgtaaacaaaacatattgtataactccgactttttctgtaacaaatggaaaatatattgttagtggttcagaagatcattgtgtctacatatgggatttacaaggg

SEQ ID NO: 78 - DNA, 240 bp, Artificial Sequence
  Synthetic DNA
cgggtcaaattcgctatctgagctgatgcattcaactatttggtctctttttaacatttattttttttattattttgaatgtagaaactttggaactactcaactggtaagttcttgaagatgtataccggtcatgtaaacaaaacatattgtataactccgactttttctgtaacaaatggaaaatatattgttagtggttcagaagatcattgtgtctacatatgggatttacaaggg

SEQ ID NO: 79 - DNA, 326 bp, Stevia rebaudiana
ggcagccattgatgatgttgttgaatgtgattaatttgaatgttataaagaatttggaaaagaaaaaggaggggacaaagttgatgaaattaggggagttatgattatgatggccatggtgattgtgatgagtggcactatgtaatctaatatttgaagatatgagaccacttgaccatgttataatcttatacaaaataattaatccctcacggtaatttttttctaatccttaaactgaaatttgaaagtaatttgagatagtgtttcccctaatttatgcttttagcatgcatttattctatcatattttctatgagaattgg

SEQ ID NO: 80 - DNA, 21 bp, Stevia rebaudiana
atgcttttagcatgcatttat

SEQ ID NO: 81 - DNA, 41 bp, Stevia rebaudiana
cccctaatttatgcttttagcatgcatttattctatcatat

SEQ ID NO: 82 - DNA, 61 bp, Stevia rebaudiana
gatagtgtttcccctaatttatgcttttagcatgcatttattctatcatattttctatgag

SEQ ID NO: 83 - DNA, 70 bp, Stevia rebaudiana
tgattttgaaaggatctgactgtatgtttatatgacatagttatgagtttgaaccccaatggctaaccct

SEQ ID NO: 84 - DNA, 21 bp, Stevia rebaudiana
tatgtttatatgacatagtta

SEQ ID NO: 85 - DNA, 41 bp, Stevia rebaudiana
gatctgactgtatgtttatatgacatagttatgagtttgaa

SEQ ID NO: 86 - DNA, 61 bp, Stevia rebaudiana
attttgaaaggatctgactgtatgtttatatgacatagttatgagtttgaaccccaatggc

SEQ ID NO: 87 - DNA, 383 bp, Stevia rebaudiana
aaggttctttatttttaaacttatgttaatttattgtatcttgaagttaatcaagagatgctctcttggagaaattttatggtcataaaacctatatcaaagagatgctctcttggtatattccatacttaaaatatctattttggaaaaaaagtgtagcatcttcctgcttttagtaggtgtcaatcattattaaatttcacaaaaccgtgcaagaatcccagtttccctatagtttgtatacgttcctgatctagtattttacttatgtttcaaatcagtccaatcatgcttgtgtccgaaaattaaaaaacaagggtattggatgccctgtaccactattattaacttttcagaaaaacgtgtagcatgtgtacataagg

SEQ ID NO: 88 - DNA, 21 bp, Stevia rebaudiana
ttgtatcttgaagttaatcaa

SEQ ID NO: 89 - DNA, 41 bp, Stevia rebaudiana
tgttaatttattgtatcttgaagttaatcaagagatgctct

SEQ ID NO: 90 - DNA, 61 bp, Stevia rebaudiana
tttaaacttatgttaatttattgtatcttgaagttaatcaagagatgctctcttggagaaa

SEQ ID NO: 91 - DNA, 297 bp, Stevia rebaudiana
taatcatccaaaccctaatctcgccaaacaaccgaataccgatccaaaccctgaaatgagcacaactcttgaacctgatcacgagaatgaagagcacaaacatgttatgacacatgtaaacgatggtttttgctacatgaaaaccctagaagacgaaacccgtttaagtgtaaatcttgaaaacacattctttgatgaagaacccctttcgtatccggatcttatggacttttctgcatcgaaaaaggacgaatacgacttctatgatgaacttgaagagttgccaatgtcttcctc

SEQ ID NO: 92 - DNA, 21 bp, Stevia rebaudiana
aaccgaataccgatccaaacc

SEQ ID NO: 93 - DNA, 41 bp, Stevia rebaudiana
ctcgccaaacaaccgaataccgatccaaaccctgaaatgag

SEQ ID NO: 94 - DNA, 61 bp, Stevia rebaudiana
aaaccctaatctcgccaaacaaccgaataccgatccaaaccctgaaatgagcacaactctt

SEQ ID NO: 95 - DNA, 390 bp, Stevia rebaudiana
cgatggtttttgctacatgaaaaccctagaagacgaaacccgtttaagtgtaaatcttgaaaacacattctttgatgaagaacccctttcgtatccggatcttatggacttttctgcatcgaaaaaggacgaatacgacttctatgatgaacttgaagagttgccaatgtcttcctcatcattcaaaagcttcatgagaagtaatttctttgaggaaagagttcttgttcaaccttattgattaagaatttaagggaagcagattatatatgtaattaaattttggtatttatactttgaacttaattaataattataataataatcccaactagaggcacttagtggagattacttatatataatactaattcaaggattattgctggt

SEQ ID NO: 96 - DNA, 21 bp, Stevia rebaudiana
acccgtttaagtgtaaatctt

SEQ ID NO: 97 - DNA, 41 bp, Stevia rebaudiana
agaagacgaaacccgtttaagtgtaaatcttgaaaacacat

SEQ ID NO: 98 - DNA, 61 bp, Stevia rebaudiana
tgaaaaccctagaagacgaaacccgtttaagtgtaaatcttgaaaacacattctttgatga

SEQ ID NO: 99 - DNA, 140 bp, Stevia rebaudiana; identical to SEQ ID NO: 72

SEQ ID NO: 100 - DNA, 38 bp, Stevia rebaudiana
attaaaattttataacaatatcatacttgaattaaaga

SEQ ID NO: 101 - DNA, 58 bp, Stevia rebaudiana
ttatttctaaattaaaattttataacaatatcatacttgaattaaagataacataata

SEQ ID NO: 102 - DNA, 78 bp, Stevia rebaudiana
aacatattttttatttctaaattaaaattttataacaatatcatacttgaattaaagataacataatatttattttta

SEQ ID NO: 103 - DNA, 288 bp, Stevia rebaudiana
atacaaaaacacaacccatatggtcaaatcaacccattcatgagtaatcgggtcaaattcgctatctgagctgatgcattcaactatttggtctctttttaacatttattttttttattattttgaatgtagaaactttggaactactcaactggtaagttcttgaagatgtataccggtcatgtaaacaaaacatattgtataactccgactttttctgtaacaaatggaaaatatattgttagtggttcagaagatcattgtgtctacatatgggatttacaaggg

SEQ ID NO: 104 - DNA, 21 bp, Stevia rebaudiana
atgagtaatcgggtcaaattc

SEQ ID NO: 105 - DNA, 41 bp, Stevia rebaudiana
caacccattcatgagtaatcgggtcaaattcgctatctgag

SEQ ID NO: 106 - DNA, 61 bp, Stevia rebaudiana
atggtcaaatcaacccattcatgagtaatcgggtcaaattcgctatctgagctgatgcatt

SEQ ID NO: 107 - DNA, 36 bp, Artificial Sequence
  Synthetic DNA
ccaattctcatagaaaatatgatagaataaatgtat

SEQ ID NO: 108 - DNA, 36 bp, Artificial Sequence
  Synthetic DNA
ccaattctcatagaaaatatgatagaataaatgcaa

SEQ ID NO: 109 - DNA, 32 bp, Artificial Sequence
  Synthetic DNA
tgattttgaaaggatctgactgtatgtttaca

SEQ ID NO: 110 - DNA, 32 bp, Artificial Sequence
  Synthetic DNA
tgattttgaaaggatctgactgtatgtttatg